European Patent Specification EP 4 185 607 B1, published September 30, 2026. Title: CO-AGONISTS AT GLP-1 AND GIP RECEPTORS SUITABLE FOR ORAL DELIVERY. Applicant: Novo Nordisk A/S. The sequence listing filed with the application follows.

SEQUENCE LISTING (48 sequences)

SEQ ID NO: 1 - protein, 39 aa, Artificial Sequence
  Synthetic
  MOD_RES (2)..(2): Aib
YXEGTFTSDYSIYLEKQAAQEFVNWLLAGGPSSGAPPPS

SEQ ID NO: 2 - protein, 39 aa, Artificial Sequence
  Synthetic
  MOD_RES (2)..(2): Aib
YXEGTFTSDYSYYLEKQAAQEFVNWLLAGGPSSGAPPPS

SEQ ID NO: 3 - protein, 39 aa, Artificial Sequence
  Synthetic
  MOD_RES (2)..(2): Aib
YXEGTFTSDYSYYLEKQAAQAFVNWLLAGGPSSGAPPPS

SEQ ID NO: 4 - protein, 39 aa, Artificial Sequence
  Synthetic
  MOD_RES (2)..(2): Aib
YXEGTFTSDYSIYLEKQAAREFVNWLLAGGPSSGAPPPS

SEQ ID NO: 5 - protein, 39 aa, Artificial Sequence
  Synthetic
  MOD_RES (2)..(2): Aib
YXEGTFTSDYSIYLEKQAAREFINWLLAGGPSSGAPPPS

SEQ ID NO: 6 - protein, 39 aa, Artificial Sequence
  Synthetic
  MOD_RES (2)..(2): Aib
YXEGTFTSDYSIYLEKQAAREFIEWLLAGGPSSGAPPPS

SEQ ID NO: 7 - protein, 39 aa, Artificial Sequence
  Synthetic
  MOD_RES (2)..(2): Aib
YXEGTFTSDYSIYLEKQAAREFIEWLLRGGPSSGAPPPS

SEQ ID NO: 8 - protein, 39 aa, Artificial Sequence
  Synthetic
  MOD_RES (2)..(2): Aib
YXEGTFTSDYSIYLEKQAAREFIEWLLRGGPESGAPPPS

SEQ ID NO: 9 - protein, 39 aa, Artificial Sequence
  Synthetic
  MOD_RES (2)..(2): Aib
YXEGTFTSDYSIALEKQAAREFINWLLAGGPSSGAPPPS

SEQ ID NO: 10 - protein, 39 aa, Artificial Sequence
  Synthetic
  MOD_RES (2)..(2): Aib
YXEGTFTSDYSILLEKQAAREFINWLLAGGPSSGAPPPS

SEQ ID NO: 11 - protein, 39 aa, Artificial Sequence
  Synthetic
YAEGTFTSDYSIYLEKQAAREFINWLLAGGPSSGAPPPS

SEQ ID NO: 12 - protein, 29 aa, Artificial Sequence
  Synthetic
  MOD_RES (2)..(2): Aib
YXEGTFTSDYSILLEKQAAREFINWLLAG

SEQ ID NO: 13 - protein, 31 aa, Artificial Sequence
  Synthetic
  MOD_RES (2)..(2): Aib
YXEGTFTSDYSILLEKQAAREFINWLLAGGP

SEQ ID NO: 14 - protein, 33 aa, Artificial Sequence
  Synthetic
  MOD_RES (2)..(2): Aib
YXEGTFTSDYSILLEKQAAREFINWLLAGGPSS

SEQ ID NO: 15 - protein, 35 aa, Artificial Sequence
  Synthetic
  MOD_RES (2)..(2): Aib
YXEGTFTSDYSILLEKQAAREFINWLLAGGPSSGA

SEQ ID NO: 16 - protein, 39 aa, Artificial Sequence
  Synthetic
  MOD_RES (2)..(2): Aib
YXEGTFTSDYSILLEKQAAREFVNWLLAGGPSSGAPPPS

SEQ ID NO: 17 - protein, 39 aa, Artificial Sequence
  Synthetic
  MOD_RES (2)..(2): Aib
YXEGTFTSDYSILLEKQAAREFIQWLLAGGPSSGAPPPS

SEQ ID NO: 18 - protein, 39 aa, Artificial Sequence
  Synthetic
  MOD_RES (2)..(2): Aib
YXEGTFTSDYSILLEKQAAQEFINWLLAGGPSSGAPPPS

SEQ ID NO: 19 - protein, 39 aa, Artificial Sequence
  Synthetic
  MOD_RES (2)..(2): Aib
YXEGTFTSDYSILLEKQAAEEFINWLLAGGPSSGAPPPS

SEQ ID NO: 20 - protein, 39 aa, Artificial Sequence
  Synthetic
  MOD_RES (2)..(2): Aib
YXEGTFTSDYSILLEKQAAHEFINWLLAGGPSSGAPPPS

SEQ ID NO: 21 - protein, 39 aa, Artificial Sequence
  Synthetic
  MOD_RES (2)..(2): Aib
YXEGTFTSDYSILLEKQAAREFIEWLLRGGPSSGAPPPS

SEQ ID NO: 22 - protein, 39 aa, Artificial Sequence
  Synthetic
  MOD_RES (2)..(2): Aib
YXEGTFTSDYSILLEKQAAREFIEWLLRGGPESGAPPPS

SEQ ID NO: 23 - protein, 39 aa, Artificial Sequence
  Synthetic
  MOD_RES (2)..(2): Aib
YXEGTFTSDYSILLEKQAAQEFIEWLLAGGPSSGAPPPS

SEQ ID NO: 24 - protein, 39 aa, Artificial Sequence
  Synthetic
  MOD_RES (2)..(2): Aib
YXEGTFTSDYSILLEKQAAHEFIEWLLAGGPSSGAPPPS

SEQ ID NO: 25 - protein, 39 aa, Artificial Sequence
  Synthetic
  MOD_RES (2)..(2): Aib
YXEGTFTSDYSILLEKQAAREFIEWLLAGGPSSGAPPPS

SEQ ID NO: 26 - protein, 39 aa, Artificial Sequence
  Synthetic
  MOD_RES (2)..(2): Aib
YXEGTVTSDYSILLEKQAAREFINWLLAGGPSSGAPPPS

SEQ ID NO: 27 - protein, 39 aa, Artificial Sequence
  Synthetic
  MOD_RES (2)..(2): Aib
YXEGTFTSDYSIILEKQAAREFINWLLAGGPSSGAPPPS

SEQ ID NO: 28 - protein, 39 aa, Artificial Sequence
  Synthetic
  MOD_RES (2)..(2): Aib
YXEGTFTSDYSIYLEEQAARKFINWLLAGGPSSGAPPPS

SEQ ID NO: 29 - protein, 39 aa, Artificial Sequence
  Synthetic
  MOD_RES (2)..(2): Aib
YXEGTFTSDYSIYLEEKAAREFINWLLAGGPSSGAPPPS

SEQ ID NO: 30 - protein, 39 aa, Artificial Sequence
  Synthetic
  MOD_RES (2)..(2): Aib
YXEGTFTSDYSILLEEQAARKFINWLLAGGPSSGAPPPS

SEQ ID NO: 31 - protein, 39 aa, Artificial Sequence
  Synthetic
  MOD_RES (2)..(2): Aib
YXEGTFTSDYSKLLEEQAAREFIEWLLAGGPSSGAPPPS

SEQ ID NO: 32 - protein, 39 aa, Artificial Sequence
  Synthetic
  MOD_RES (2)..(2): Aib
YXEGTFTSDYSKYLEEQAAREFINWLLAGGPSSGAPPPS

SEQ ID NO: 33 - protein, 39 aa, Artificial Sequence
  Synthetic
  MOD_RES (2)..(2): Aib
YXEGTFTSDYSIYLEEQAAREFINWLLAGGPSKGAPPPS

SEQ ID NO: 34 - protein, 39 aa, Artificial Sequence
  Synthetic
  MOD_RES (2)..(2): Aib
YXEGTFTSDYSILLEEQAAREFIEWLLAGGPSKGAPPPS

SEQ ID NO: 35 - protein, 39 aa, Artificial Sequence
  Synthetic
  MOD_RES (2)..(2): Aib
YXEGTFTSDYSILLEEQAAREFINWLLAGGPSKGAPPPS

SEQ ID NO: 36 - protein, 39 aa, Artificial Sequence
  Synthetic
  MISC_FEATURE (2)..(2): Xaa is Aib or Ala
  MISC_FEATURE (6)..(6): Xaa is Phe or Val
  MISC_FEATURE (12)..(12): Xaa is Ile or Tyr
  MISC_FEATURE (13)..(13): Xaa is Tyr, Ala, Leu or Ile
  MISC_FEATURE (16)..(16): Xaa is Lys or Glu
  MISC_FEATURE (20)..(20): Xaa is Gln, Arg, Glu or His
  MISC_FEATURE (21)..(21): Xaa is Ala or Glu
  MISC_FEATURE (23)..(23): Xaa is Ile or Val
  MISC_FEATURE (24)..(24): Xaa is Glu, Gln or Asn
  MISC_FEATURE (28)..(28): Xaa is Ala or Arg
  MISC_FEATURE (32)..(32): Xaa is Glu, Ser or absent
  MISC_FEATURE (33)..(33): Xaa is Ser, Lys or absent
  MISC_FEATURE (34)..(34): Xaa is Gly or absent
  MISC_FEATURE (35)..(35): Xaa is Ala or absent
  MISC_FEATURE (36)..(36): Xaa is Pro or absent
  MISC_FEATURE (37)..(37): Xaa is Pro or absent
  MISC_FEATURE (38)..(38): Xaa is Pro or absent
  MISC_FEATURE (39)..(39): Xaa is Ser or absent
YXEGTXTSDYSXXLEXQAAXXFXXWLLXGGPXXXXXXXX

SEQ ID NO: 37 - protein, 39 aa, Artificial Sequence
  Synthetic
  MISC_FEATURE (2)..(2): Xaa is Aib or Ala
  MISC_FEATURE (6)..(6): Xaa is Phe or Val
  MISC_FEATURE (12)..(12): Xaa is Ile or Tyr
  MISC_FEATURE (13)..(13): Xaa is Tyr, Ala, Leu or Ile
  MISC_FEATURE (16)..(16): Xaa is Lys or Glu
  MISC_FEATURE (20)..(20): Xaa is Gln, Arg, Glu or His
  MISC_FEATURE (21)..(21): Xaa is Ala or Glu
  MISC_FEATURE (23)..(23): Xaa is Ile or Val
  MISC_FEATURE (24)..(24): Xaa is Glu, Gln or Asn
  MISC_FEATURE (28)..(28): Xaa is Ala or Arg
YXEGTXTSDYSXXLEXQAAXXFXXWLLXGGPSSGAPPPS

SEQ ID NO: 38 - protein, 39 aa, Artificial Sequence
  Synthetic
  MISC_FEATURE (2)..(2): Xaa is Aib or Ala
  MISC_FEATURE (6)..(6): Xaa is Phe or Val
  MISC_FEATURE (12)..(12): Xaa is Ile or Tyr
  MISC_FEATURE (13)..(13): Xaa is Tyr, Ala, Leu or Ile
  MISC_FEATURE (16)..(16): Xaa is Lys or Glu
  MISC_FEATURE (20)..(20): Xaa is Gln, Arg, Glu or His
  MISC_FEATURE (21)..(21): Xaa is Ala or Glu
  MISC_FEATURE (23)..(23): Xaa is Ile or Val
  MISC_FEATURE (24)..(24): Xaa is Glu, Gln or Asn
  MISC_FEATURE (28)..(28): Xaa is Ala or Arg
YXEGTXTSDYSXXLEXQAAXXFXXWLLXGGPESGAPPPS

SEQ ID NO: 39 - protein, 39 aa, Artificial Sequence
  Synthetic
  MISC_FEATURE (2)..(2): Xaa is Aib or Ala
  MISC_FEATURE (6)..(6): Xaa is Phe or Val
  MISC_FEATURE (12)..(12): Xaa is Ile or Tyr
  MISC_FEATURE (13)..(13): Xaa is Tyr, Ala, Leu or Ile
  MISC_FEATURE (16)..(16): Xaa is Lys or Glu
  MISC_FEATURE (20)..(20): Xaa is Gln, Arg, Glu or His
  MISC_FEATURE (21)..(21): Xaa is Ala or Glu
  MISC_FEATURE (23)..(23): Xaa is Ile or Val
  MISC_FEATURE (24)..(24): Xaa is Glu, Gln or Asn
  MISC_FEATURE (28)..(28): Xaa is Ala or Arg
YXEGTXTSDYSXXLEXQAAXXFXXWLLXGGPSKGAPPPS

SEQ ID NO: 40 - protein, 4 aa, Artificial Sequence
  Synthetic
SSGA

SEQ ID NO: 41 - protein, 4 aa, Artificial Sequence
  Synthetic
ESGA

SEQ ID NO: 42 - protein, 4 aa, Artificial Sequence
  Synthetic
SKGA

SEQ ID NO: 43 - protein, 12 aa, Artificial Sequence
  Synthetic
LLEKQAAREFIN

SEQ ID NO: 44 - protein, 12 aa, Artificial Sequence
  Synthetic
LLEKQAAREFIE

SEQ ID NO: 45 - protein, 12 aa, Artificial Sequence
  Synthetic
LLEKQAAQEFIE

SEQ ID NO: 46 - protein, 12 aa, Artificial Sequence
  Synthetic
LLEEQAAREFIE

SEQ ID NO: 47 - protein, 39 aa, Artificial Sequence
  Synthetic
  MOD_RES (2)..(2): Aib
  MISC_FEATURE (2)..(2): Xaa is Aib or Ala
  MISC_FEATURE (6)..(6): Xaa is Phe or Val
  MISC_FEATURE (12)..(12): Xaa is Ile or Tyr
  MISC_FEATURE (13)..(13): Xaa is Tyr, Ala, Leu or Ile
  MISC_FEATURE (16)..(16): Xaa is Lys or Glu
  MISC_FEATURE (20)..(20): Xaa is Gln, Arg, Glu or His
  MISC_FEATURE (21)..(21): Xaa is Ala or Glu
  MISC_FEATURE (23)..(23): Xaa is Ile or Val
  MISC_FEATURE (24)..(24): Xaa is Glu, Gln or Asn
  MISC_FEATURE (28)..(28): Xaa is Ala or Arg
  MISC_FEATURE (30)..(30): Xaa is Gly or absent
  MISC_FEATURE (31)..(31): Xaa is Pro or absent
  MISC_FEATURE (32)..(32): Xaa is Glu, Ser or absent
  MISC_FEATURE (33)..(33): Xaa is Ser, Lys or absent
  MISC_FEATURE (34)..(34): Xaa is Gly or absent
  MISC_FEATURE (35)..(35): Xaa is Ala or absent
  MISC_FEATURE (36)..(36): Xaa is Pro or absent
  MISC_FEATURE (37)..(37): Xaa is Pro or absent
  MISC_FEATURE (38)..(38): Xaa is Pro or absent
  MISC_FEATURE (39)..(39): Xaa is Ser or absent
YXEGTXTSDYSXXLEXQAAXXFXXWLLXGXXXXXXXXXX

SEQ ID NO: 48 - protein, 29 aa, Homo sapiens
HSQGTFTSDYSKYLDSRRAQDFVQWLMNT